European Patent Specification EP 4 323 388 B1, published January 29, 2025. Title: N-terminal capping modules of ankyrin repeat domains. Applicant: Athebio AG. The sequence listing filed with the application follows.

SEQUENCE LISTING (100 sequences)

SEQ ID NO: 1 - protein, 30 aa, Artificial Sequence
  Synthetic construct
DLGKKLLEAARAGQDDEVRILMANGADVNA

SEQ ID NO: 2 - protein, 30 aa, Artificial Sequence
  Synthetic construct
DLGKKLLEAARAGQDDEVRELLKAGADVNA

SEQ ID NO: 3 - protein, 30 aa, Artificial Sequence
  Synthetic construct
DLGKKLLEAARAGQDDEVRILLKAGADVNA

SEQ ID NO: 4 - protein, 30 aa, Artificial Sequence
  Synthetic construct
DLDKKLLEAARAGQDDEVRILMANGADVNA

SEQ ID NO: 5 - protein, 30 aa, Artificial Sequence
  Synthetic construct
DLGKKLLEAARAGQDDEVRILIANGAPFTT

SEQ ID NO: 6 - protein, 30 aa, Artificial Sequence
  Synthetic construct
DLGKKLLEAARAGQDDEVRELTKAGADVNA

SEQ ID NO: 7 - protein, 30 aa, Artificial Sequence
  Synthetic construct
DLGKKLLEAARAGQDDEVHILIANGADVNA

SEQ ID NO: 8 - protein, 30 aa, Artificial Sequence
  Synthetic construct
DLGKKLLQAARAGQLDEVRELLKAGADVNA

SEQ ID NO: 9 - protein, 30 aa, Artificial Sequence
  Synthetic construct
DLGKKLLKAARAGQKDEVKILMENGADVNA

SEQ ID NO: 10 - protein, 30 aa, Artificial Sequence
  Synthetic construct
DLGKKLLEAARAGQDDEVRILMALGADVNA

SEQ ID NO: 11 - protein, 30 aa, Artificial Sequence
  Synthetic construct
DLGKKLLEAARAGQIDEVRELLKLGADVNA

SEQ ID NO: 12 - protein, 30 aa, Artificial Sequence
  Synthetic construct
DLDKKLLEAARAGQLDEVRELTKLGADVNA

SEQ ID NO: 13 - protein, 30 aa, Artificial Sequence
  Synthetic construct
DLGKKLLEAARAGQVDEVRELIKLGADVNA

SEQ ID NO: 14 - protein, 30 aa, Artificial Sequence
  Synthetic construct
DLDKKLLEAAAAGQIDAVRELLKLGADVNA

SEQ ID NO: 15 - protein, 30 aa, Artificial Sequence
  Synthetic construct
DLAKKLLEAAAAGQLDAVRELVKLGADVNA

SEQ ID NO: 16 - protein, 30 aa, Artificial Sequence
  Synthetic construct
DLGKKLLEAAAAGQVDAVRELIKLGADVNA

SEQ ID NO: 17 - protein, 30 aa, Artificial Sequence
  Synthetic construct
DLAKKLLEAAAAGQIDAVRELAKLGADVNA

SEQ ID NO: 18 - protein, 30 aa, Artificial Sequence
  Synthetic construct
DLAKKLLAAAAAGQLEAVEQLLKLGADVNA

SEQ ID NO: 19 - protein, 30 aa, Artificial Sequence
  Synthetic construct
DLGKKLLAAAAAGQVEAVEQLIKLGADVNA

SEQ ID NO: 20 - protein, 30 aa, Artificial Sequence
  Synthetic construct
DLGKKLLEAAAAGQLDEVRILIALGADVNA

SEQ ID NO: 21 - protein, 30 aa, Artificial Sequence
  Synthetic construct
DLGKKLLEAAAAGQLDEVKELIALGADVNA

SEQ ID NO: 22 - protein, 30 aa, Artificial Sequence
  Synthetic construct
DLGKKLLEAARAGQLDEVRELLKLGADVNA

SEQ ID NO: 23 - protein, 30 aa, Artificial Sequence
  Synthetic construct
DLGKKLLEAAEAGQVDEVKELLKLGADVNA

SEQ ID NO: 24 - protein, 30 aa, Artificial Sequence
  Synthetic construct
DLGKKLLEAARAGQLDEVRILLKLGADVNA

SEQ ID NO: 25 - protein, 30 aa, Artificial Sequence
  Synthetic construct
DLGKKLLEAAEAGQVDEVKILLKLGADVNA

SEQ ID NO: 26 - protein, 30 aa, Artificial Sequence
  Synthetic construct
DLGKKLLEAAAAGQVDEVRELIKLGADVNA

SEQ ID NO: 27 - protein, 30 aa, Artificial Sequence
  Synthetic construct
DLGKKLLEAAAAGQVDEVKELIKLGADVNA

SEQ ID NO: 28 - protein, 30 aa, Artificial Sequence
  Synthetic construct
DLGKKLLEAARAGQLDEVRILIKLGADVNA

SEQ ID NO: 29 - protein, 30 aa, Artificial Sequence
  Synthetic construct
DLGKKLLEAARAGQLDEVKILIKLGADVNA

SEQ ID NO: 30 - protein, 30 aa, Artificial Sequence
  Synthetic construct
DLGKKLLEAAEAGQLDEVRELLALGADVNA

SEQ ID NO: 31 - protein, 30 aa, Artificial Sequence
  Synthetic construct
DLGKKLLEAAEAGQLDEVKELLALGADVNA

SEQ ID NO: 32 - protein, 30 aa, Artificial Sequence
  Synthetic construct
DLGKKLLEAAAAGQVDEVKELIALGADVNA

SEQ ID NO: 33 - protein, 30 aa, Artificial Sequence
  Synthetic construct
DLGKKLLEAARAGQIDEVKILLALGADVNA

SEQ ID NO: 34 - protein, 30 aa, Artificial Sequence
  Synthetic construct
DLGKKLLEAAAAGQIDEVRELIALGADVNA

SEQ ID NO: 35 - protein, 30 aa, Artificial Sequence
  Synthetic construct
DLGKKLLEAAAAGQIDEVKELIALGADVNA

SEQ ID NO: 36 - protein, 30 aa, Artificial Sequence
  Synthetic construct
DLGKKLLEAAEAGQIDEVRILIALGADVNA

SEQ ID NO: 37 - protein, 30 aa, Artificial Sequence
  Synthetic construct
DLGKKLLEAAEAGQIDEVKILIALGADVNA

SEQ ID NO: 38 - protein, 30 aa, Artificial Sequence
  Synthetic construct
  VARIANT 1: Xaa is selected from the group consisting of G, D, A, E, N, Q, S, T, K, R, H and C
  VARIANT 2: Xaa is selected from the group consisting of L, Q, E, M, K, R and C
  VARIANT 3: Xaa is selected from the group consisting of G, A, D, S and C
  VARIANT 4: Xaa is selected from the group consisting of Q, N, S, T, A, D, E, K, R, H and C
  VARIANT 5: Xaa is selected from the group consisting of Q, N, S, T, A, D, E, K, R, H and C
  VARIANT 6: Xaa is selected from the group consisting of L, A, N, S, D and C
  VARIANT 7: Xaa is selected from the group consisting of L, I, V, A, N, T, S, D and C
  VARIANT 8: Xaa is selected from the group consisting of Q, N, S, T, A, D, E, K, R, H and C
  VARIANT 10: Xaa is selected from the group consisting of A, V, S and C
  VARIANT 11: Xaa is selected from the group consisting of R, A, L, S, Q, K, H, D, E, C, T, N, F, W and Y
  VARIANT 12: Xaa is selected from the group consisting of Q, N, S, T, A, D, E, K, R, H and C
  VARIANT 13: Xaa is selected from the group consisting of G and C
  VARIANT 14: Xaa is selected from the group consisting of Q, N, S, T, A, D, E, K, R, H and C
  VARIANT 15: Xaa is selected from the group consisting of D, L, M, I, T, A, V, S, N, Q, K, R, E and C
  VARIANT 16: Xaa is selected from the group consisting of Q, N, S, T, A, D, E, K, R, H and C
  VARIANT 17: Xaa is selected from the group consisting of Q, N, S, T, A, D, E, K, R, H and C
  VARIANT 18: Xaa is selected from the group consisting of L, I, V, T, A, S and C
  VARIANT 19: Xaa is selected from the group consisting of Q, N, S, T, A, D, E, K, R, H and C
  VARIANT 20: Xaa is selected from the group consisting of E, Q, N, K, R, A, D, T, S, H, I, V and C
  VARIANT 21: Xaa is selected from the group consisting of L, N, S, A and C
  VARIANT 22: Xaa is selected from the group consisting of L, I, A, V, M, T, S, N and C
  VARIANT 23: Xaa is selected from the group consisting of K, R, S, Q, N, A, E, D, H and C
  VARIANT 24: Xaa is selected from the group consisting of A, K, R, H, L, I, V, C and G
  VARIANT 27: Xaa is selected from the group consisting of D, N and C
  VARIANT 28: Xaa is selected from the group consisting of V, T, S, P, A and C
  VARIANT 29: Xaa is selected from the group consisting of N, D and C
  VARIANT 30: Xaa is selected from the group consisting of A and C
XXXXXXXXAXXXXXXXXXXXXXXXGAXXXX

SEQ ID NO: 39 - protein, 33 aa, Artificial Sequence
  Synthetic construct
  VARIANT 1: Xaa can be any naturally occuring amino acid residue
  VARIANT 3: Xaa can be any naturally occuring amino acid residue
  VARIANT 4: Xaa can be any naturally occuring amino acid residue
  VARIANT 6: Xaa can be any naturally occuring amino acid residue
  VARIANT 13: Xaa can be any naturally occuring amino acid residue
  VARIANT 14: Xaa can be any naturally occuring amino acid residue
  VARIANT 15: Xaa can be any naturally occuring amino acid residue
  VARIANT 17: Xaa can be any naturally occuring amino acid residue
  VARIANT 18: Xaa can be any naturally occuring amino acid residue
  VARIANT 19: Xaa can be any naturally occuring amino acid residue
  VARIANT 22: Xaa can be any naturally occuring amino acid residue
  VARIANT 26: Xaa can be any naturally occuring amino acid residue
  VARIANT 27: Xaa can be any naturally occuring amino acid residue
XDXXGXTPLHLAXXXGXXXVVXLLLXXGADVNA

SEQ ID NO: 40 - protein, 33 aa, Artificial Sequence
  Synthetic construct
  VARIANT 1: Xaa can be any naturally occuring amino acid residue
  VARIANT 3: Xaa can be any naturally occuring amino acid residue
  VARIANT 4: Xaa can be any naturally occuring amino acid residue
  VARIANT 6: Xaa can be any naturally occuring amino acid residue
  VARIANT 14: Xaa can be any naturally occuring amino acid residue
  VARIANT 15: Xaa can be any naturally occuring amino acid residue
  VARIANT 27: Xaa can be any naturally occuring amino acid residue
XDXXGXTPLHLAAXXGHLEIVEVLLKXGADVNA

SEQ ID NO: 41 - protein, 33 aa, Artificial Sequence
  Synthetic construct
  VARIANT 2: Xaa can be any naturally occuring amino acid residue
  VARIANT 3: Xaa can be any naturally occuring amino acid residue
  VARIANT 4: Xaa can be any naturally occuring amino acid residue
  VARIANT 6: Xaa can be any naturally occuring amino acid residue
  VARIANT 11: Xaa can be any naturally occuring amino acid residue
  VARIANT 14: Xaa can be any naturally occuring amino acid residue
  VARIANT 15: Xaa can be any naturally occuring amino acid residue
  VARIANT 27: Xaa can be any naturally occuring amino acid residue
SXXXGXTPLHXAAXXGHLEIVDVLLAXGADVNA

SEQ ID NO: 42 - protein, 33 aa, Artificial Sequence
  Synthetic construct
  VARIANT 1: Xaa can be any naturally occuring amino acid residue
  VARIANT 3: Xaa can be any naturally occuring amino acid residue
  VARIANT 4: Xaa can be any naturally occuring amino acid residue
  VARIANT 6: Xaa can be any naturally occuring amino acid residue
  VARIANT 14: Xaa can be any naturally occuring amino acid residue
  VARIANT 15: Xaa can be any naturally occuring amino acid residue
XDXXGXTPLHLAAXXGHLEIVEVLLKNGADVNA

SEQ ID NO: 43 - protein, 33 aa, Artificial Sequence
  Synthetic construct
  VARIANT 3: Xaa can be any naturally occuring amino acid residue
  VARIANT 4: Xaa can be any naturally occuring amino acid residue
  VARIANT 6: Xaa can be any naturally occuring amino acid residue
  VARIANT 14: Xaa can be any naturally occuring amino acid residue
  VARIANT 15: Xaa can be any naturally occuring amino acid residue
KDXXGXTPLHLAAXXGHLEIVEVLLKAGADVNA

SEQ ID NO: 44 - protein, 33 aa, Artificial Sequence
  Synthetic construct
  VARIANT 1: Xaa can be any naturally occuring amino acid residue
  VARIANT 3: Xaa can be any naturally occuring amino acid residue
  VARIANT 4: Xaa can be any naturally occuring amino acid residue
  VARIANT 6: Xaa can be any naturally occuring amino acid residue
  VARIANT 11: Xaa can be any naturally occuring amino acid residue
  VARIANT 14: Xaa can be any naturally occuring amino acid residue
  VARIANT 15: Xaa can be any naturally occuring amino acid residue
  VARIANT 27: Xaa can be any naturally occuring amino acid residue
XDXXGXTPLHXAAXXGHLEVVKLLLEXGADVNA

SEQ ID NO: 45 - protein, 28 aa, Artificial Sequence
  Synthetic construct
QDKFGKTAFDISIDNGNEDLAEILQKLN

SEQ ID NO: 46 - protein, 28 aa, Artificial Sequence
  Synthetic construct
QDKFGKTAFDISIDNGNEDLAEILQKAA

SEQ ID NO: 47 - protein, 28 aa, Artificial Sequence
  Synthetic construct
QDKFGKTPFDLAIDNGNEDIAEVLQKAA

SEQ ID NO: 48 - protein, 28 aa, Artificial Sequence
  Synthetic construct
QDKFGKTPFDLAIREGHEDIAEVLQKAA

SEQ ID NO: 49 - protein, 28 aa, Artificial Sequence
  Synthetic construct
QDKSGKTPADLAADAGHEDIAEVLQKAA

SEQ ID NO: 50 - protein, 28 aa, Artificial Sequence
  Synthetic construct
QDSAGKTPADLAADAGHEEIAEVLQKAA

SEQ ID NO: 51 - protein, 28 aa, Artificial Sequence
  Synthetic construct
QDKAGLTPADLAADAGHEEIAEVLQKAA

SEQ ID NO: 52 - protein, 28 aa, Artificial Sequence
  Synthetic construct
QDSLGKTPADLAALAGHEEIAEVLQKAA

SEQ ID NO: 53 - protein, 28 aa, Artificial Sequence
  Synthetic construct
QDKAGQTPADLAADAGHEEIAEVLQKAA

SEQ ID NO: 54 - protein, 28 aa, Artificial Sequence
  Synthetic construct
  VARIANT 3: Xaa can be any naturally occuring amino acid residue
  VARIANT 4: Xaa can be any naturally occuring amino acid residue
  VARIANT 6: Xaa can be any naturally occuring amino acid residue
  VARIANT 14: Xaa can be any naturally occuring amino acid residue
QDXXGXTPADLAAXAGHEEIAEVLQKAA

SEQ ID NO: 55 - protein, 28 aa, Artificial Sequence
  Synthetic construct
QDKSGKTPADLAARAGHQDIAEVLQKAA

SEQ ID NO: 56 - protein, 28 aa, Artificial Sequence
  Synthetic construct
QDKFGKTAEDLAKDNGNQDIADLLEKAL

SEQ ID NO: 57 - protein, 27 aa, Artificial Sequence
  Synthetic construct
QDKFGKTAFDISIDNGNEELAKVLQDH

SEQ ID NO: 58 - protein, 103 aa, Artificial Sequence
  Synthetic construct
MRGSHHHHHHGSDLGKKLLEAAAAGQLDEVKELIAAGADVNAKDKDGYTPLHLAAREGHLEIVEVLLKAGADVNAQDKFGKTAFDISIDNGNEDLAEILQKLN

SEQ ID NO: 59 - protein, 103 aa, Artificial Sequence
  Synthetic construct
MRGSHHHHHHGSDLGKKLLEAAAAGQLDEVKELIALGADVNAKDKDGYTPLHLAAREGHLEIVEVLLKAGADVNAQDKFGKTAFDISIDNGNEDLAEILQKLN

SEQ ID NO: 60 - protein, 103 aa, Artificial Sequence
  Synthetic construct
MRGSHHHHHHGSDLGKKLLEAAAAGQLDEVKELIAGGADVNAKDKDGYTPLHLAAREGHLEIVEVLLKAGADVNAQDKFGKTAFDISIDNGNEDLAEILQKLN

SEQ ID NO: 61 - protein, 103 aa, Artificial Sequence
  Synthetic construct
MRGSHHHHHHGSDLGKKLLEAAAAGQLDEVKELIAVGADVNAKDKDGYTPLHLAAREGHLEIVEVLLKAGADVNAQDKFGKTAFDISIDNGNEDLAEILQKLN

SEQ ID NO: 62 - protein, 103 aa, Artificial Sequence
  Synthetic construct
MRGSHHHHHHGSDLGKKLLEAAAAGQLDEVKELIAEGADVNAKDKDGYTPLHLAAREGHLEIVEVLLKAGADVNAQDKFGKTAFDISIDNGNEDLAEILQKLN

SEQ ID NO: 63 - protein, 103 aa, Artificial Sequence
  Synthetic construct
MRGSHHHHHHGSDLGKKLLEAAAAGQLDEVKELIANGADVNAKDKDGYTPLHLAAREGHLEIVEVLLKAGADVNAQDKFGKTAFDISIDNGNEDLAEILQKLN

SEQ ID NO: 64 - protein, 103 aa, Artificial Sequence
  Synthetic construct
MRGSHHHHHHGSDLGKKLLEAAAAGQLDEVKELIAQGADVNAKDKDGYTPLHLAAREGHLEIVEVLLKAGADVNAQDKFGKTAFDISIDNGNEDLAEILQKLN

SEQ ID NO: 65 - protein, 103 aa, Artificial Sequence
  Synthetic construct
MRGSHHHHHHGSDLGKKLLEAAAAGQLDEVKELIASGADVNAKDKDGYTPLHLAAREGHLEIVEVLLKAGADVNAQDKFGKTAFDISIDNGNEDLAEILQKLN

SEQ ID NO: 66 - protein, 136 aa, Artificial Sequence
  Synthetic construct
MRGSHHHHHHGSDLGKKLLEAARAGQDDEVRELLKAGADVNAKDYFSHTPLHLAARNGHLKIVEVLLKAGADVNAKDFAGKTPLHLAANEGHLEIVEVLLKAGADVNAQDIFGKTPADIAADAGHEDIAEVLQKAA

SEQ ID NO: 67 - protein, 136 aa, Artificial Sequence
  Synthetic construct
MRGSHHHHHHGSDLGKKLLEAARAGQDDEVRELLKLGADVNAKDYFSHTPLHLAARNGHLKIVEVLLKAGADVNAKDFAGKTPLHLAANEGHLEIVEVLLKAGADVNAQDIFGKTPADIAADAGHEDIAEVLQKAA

SEQ ID NO: 68 - protein, 136 aa, Artificial Sequence
  Synthetic construct
MRGSHHHHHHGSDLDKKLLEAARAGQDDEVRILMANGADVNARDSTGWTPLHLAAPWGHPEIVEVLLKNGADVNAADFQGWTPLHLAAAVGHLEIVEVLLKYGADVNAQDKFGKTAFDISIDNGNEDLAEILQKAA

SEQ ID NO: 69 - protein, 136 aa, Artificial Sequence
  Synthetic construct
MRGSHHHHHHGSDLDKKLLEAARAGQDDEVRILMALGADVNARDSTGWTPLHLAAPWGHPEIVEVLLKNGADVNAADFQGWTPLHLAAAVGHLEIVEVLLKYGADVNAQDKFGKTAFDISIDNGNEDLAEILQKAA

SEQ ID NO: 70 - protein, 136 aa, Artificial Sequence
  Synthetic construct
MRGSHHHHHHGSDLGKKLLEAARAGQDDEVRILMANGADVNAKDEYGLTPLYLATAHGHLEIVEVLLKNGADVNAVDAIGFTPLHLAAFIGHLEIAEVLLKHGADVNAQDKFGKTAFDISIGNGNEDLAEILQKLN

SEQ ID NO: 71 - protein, 136 aa, Artificial Sequence
  Synthetic construct
MRGSHHHHHHGSDLGKKLLEAARAGQDDEVRILMALGADVNAKDEYGLTPLYLATAHGHLEIVEVLLKNGADVNAVDAIGFTPLHLAAFIGHLEIAEVLLKHGADVNAQDKFGKTAFDISIGNGNEDLAEILQKLN

SEQ ID NO: 72 - protein, 169 aa, Artificial Sequence
  Synthetic construct
MRGSHHHHHHGSDLGKKLLQAARAGQLDEVRELLKAGADVNAKDREGITPLHLAAQHGHLEIVEVLLKAGADVNAKDVWGRTPLHLAAQWGHLEIVEVLLKAGADVNAKDLAGATPLHVAALYGHLEIVEVLLKAGADVNAQDKSGKTPADLAARAGHQDIAEVLQKAA

SEQ ID NO: 73 - protein, 169 aa, Artificial Sequence
  Synthetic construct
MRGSHHHHHHGSDLGKKLLQAARAGQLDEVRELLKLGADVNAKDREGITPLHLAAQHGHLEIVEVLLKAGADVNAKDVWGRTPLHLAAQWGHLEIVEVLLKAGADVNAKDLAGATPLHVAALYGHLEIVEVLLKAGADVNAQDKSGKTPADLAARAGHQDIAEVLQKAA

SEQ ID NO: 74 - protein, 136 aa, Artificial Sequence
  Synthetic construct
MRGSHHHHHHGSDLGKKLLEAAAAGQDDEVKELIALGADVNAKDYFSHTPLHLAARNGHLKIVEVLLKAGADVNAKDFAGKTPLHLAANEGHLEIVEVLLKAGADVNAQDIFGKTPADIAADAGHEDIAEVLQKAA

SEQ ID NO: 75 - protein, 136 aa, Artificial Sequence
  Synthetic construct
MRGSHHHHHHGSDLGKKLLEAAAAGQLDEVKELIALGADVNAKDYFSHTPLHLAARNGHLKIVEVLLKAGADVNAKDFAGKTPLHLAANEGHLEIVEVLLKAGADVNAQDIFGKTPADIAADAGHEDIAEVLQKAA

SEQ ID NO: 76 - protein, 136 aa, Artificial Sequence
  Synthetic construct
MRGSHHHHHHGSDLGKKLLEAAAAGQVDEVKELIALGADVNAKDYFSHTPLHLAARNGHLKIVEVLLKAGADVNAKDFAGKTPLHLAANEGHLEIVEVLLKAGADVNAQDIFGKTPADIAADAGHEDIAEVLQKAA

SEQ ID NO: 77 - protein, 136 aa, Artificial Sequence
  Synthetic construct
MRGSHHHHHHGSDLGKKLLEAAAAGQIDEVKELIALGADVNAKDYFSHTPLHLAARNGHLKIVEVLLKAGADVNAKDFAGKTPLHLAANEGHLEIVEVLLKAGADVNAQDIFGKTPADIAADAGHEDIAEVLQKAA

SEQ ID NO: 78 - protein, 103 aa, Artificial Sequence
  Synthetic construct
MRGSHHHHHHGSDLGKKLLEAARAGQLDEVKELIAAGADVNAKDKDGYTPLHLAAREGHLEIVEVLLKAGADVNAQDKFGKTAFDISIDNGNEDLAEILQKLN

SEQ ID NO: 79 - protein, 103 aa, Artificial Sequence; identical to SEQ ID NO: 58
  Synthetic construct

SEQ ID NO: 80 - protein, 103 aa, Artificial Sequence
  Synthetic construct
MRGSHHHHHHGSDLGKKLLEAAKAGQLDEVKELIAAGADVNAKDKDGYTPLHLAAREGHLEIVEVLLKAGADVNAQDKFGKTAFDISIDNGNEDLAEILQKLN

SEQ ID NO: 81 - protein, 103 aa, Artificial Sequence
  Synthetic construct
MRGSHHHHHHGSDLGKKLLEAAEAGQLDEVKELIAAGADVNAKDKDGYTPLHLAAREGHLEIVEVLLKAGADVNAQDKFGKTAFDISIDNGNEDLAEILQKLN

SEQ ID NO: 82 - protein, 103 aa, Artificial Sequence
  Synthetic construct
MRGSHHHHHHGSDLGKKLLEAAQAGQLDEVKELIAAGADVNAKDKDGYTPLHLAAREGHLEIVEVLLKAGADVNAQDKFGKTAFDISIDNGNEDLAEILQKLN

SEQ ID NO: 83 - protein, 103 aa, Artificial Sequence
  Synthetic construct
MRGSHHHHHHGSDLGKKLLEAALAGQLDEVKELIAAGADVNAKDKDGYTPLHLAAREGHLEIVEVLLKAGADVNAQDKFGKTAFDISIDNGNEDLAEILQKLN

SEQ ID NO: 84 - protein, 103 aa, Artificial Sequence
  Synthetic construct
MRGSHHHHHHGSDLGKKLLAAARAGQLDEVRELIKAGADVNAKDKDGYTPLHLAAREGHLEIVEVLLKAGADVNAQDKFGKTAFDISIDNGNEDLAEILQKLN

SEQ ID NO: 85 - protein, 103 aa, Artificial Sequence
  Synthetic construct
MRGSHHHHHHGSDLGKKLLAAARAGQLDEVKELIKAGADVNAKDKDGYTPLHLAAREGHLEIVEVLLKAGADVNAQDKFGKTAFDISIDNGNEDLAEILQKLN

SEQ ID NO: 86 - protein, 103 aa, Artificial Sequence
  Synthetic construct
MRGSHHHHHHGSDLGKKLLAAARAGQLDEVRELIAKGADVNAKDKDGYTPLHLAAREGHLEIVEVLLKAGADVNAQDKFGKTAFDISIDNGNEDLAEILQKLN

SEQ ID NO: 87 - protein, 103 aa, Artificial Sequence
  Synthetic construct
MRGSHHHHHHGSDLGKKLLAAARAGQLDEVKELIAKGADVNAKDKDGYTPLHLAAREGHLEIVEVLLKAGADVNAQDKFGKTAFDISIDNGNEDLAEILQKLN

SEQ ID NO: 88 - protein, 136 aa, Artificial Sequence
  Synthetic construct
MRGSHHHHHHGSDLGKKLLAAARAGQLDEVRELIKAGADVNAKDYFSHTPLHLAARNGHLKIVEVLLKAGADVNAKDFAGKTPLHLAANEGHLEIVEVLLKAGADVNAQDIFGKTPADIAADAGHEDIAEVLQKAA

SEQ ID NO: 89 - protein, 136 aa, Artificial Sequence
  Synthetic construct
MRGSHHHHHHGSDLGKKLLAAARAGQLDEVKELIKAGADVNAKDYFSHTPLHLAARNGHLKIVEVLLKAGADVNAKDFAGKTPLHLAANEGHLEIVEVLLKAGADVNAQDIFGKTPADIAADAGHEDIAEVLQKAA

SEQ ID NO: 90 - protein, 136 aa, Artificial Sequence
  Synthetic construct
MRGSHHHHHHGSDLGKKLLAAARAGQLDEVRELIAKGADVNAKDYFSHTPLHLAARNGHLKIVEVLLKAGADVNAKDFAGKTPLHLAANEGHLEIVEVLLKAGADVNAQDIFGKTPADIAADAGHEDIAEVLQKAA

SEQ ID NO: 91 - protein, 136 aa, Artificial Sequence
  Synthetic construct
MRGSHHHHHHGSDLGKKLLAAARAGQLDEVKELIAKGADVNAKDYFSHTPLHLAARNGHLKIVEVLLKAGADVNAKDFAGKTPLHLAANEGHLEIVEVLLKAGADVNAQDIFGKTPADIAADAGHEDIAEVLQKAA

SEQ ID NO: 92 - protein, 136 aa, Artificial Sequence
  Synthetic construct
MRGSHHHHHHGSDLGKKLLAAARAGQLDEVRELIKAGADVNAKDEYGLTPLYLATAHGHLEIVEVLLKAGADVNAVDAIGFTPLHLAAFIGHLEIAEVLLKAGADVNAQDKFGKTPADIAAGAGNEDIAEVLQKLN

SEQ ID NO: 93 - protein, 136 aa, Artificial Sequence
  Synthetic construct
MRGSHHHHHHGSDLGKKLLAAARAGQLDEVKELIKAGADVNAKDEYGLTPLYLATAHGHLEIVEVLLKAGADVNAVDAIGFTPLHLAAFIGHLEIAEVLLKAGADVNAQDKFGKTPADIAAGAGNEDIAEVLQKLN

SEQ ID NO: 94 - protein, 103 aa, Artificial Sequence; identical to SEQ ID NO: 84
  Synthetic construct

SEQ ID NO: 95 - protein, 103 aa, Artificial Sequence
  Synthetic construct
MRGSHHHHHHGSDLGKKLLAAARAGQLDEVRELIAAGADVNAKDKDGYTPLHLAAREGHLEIVEVLLKAGADVNAQDKFGKTAFDISIDNGNEDLAEILQKLN

SEQ ID NO: 96 - protein, 136 aa, Artificial Sequence; identical to SEQ ID NO: 88
  Synthetic construct

SEQ ID NO: 97 - protein, 136 aa, Artificial Sequence
  Synthetic construct
MRGSHHHHHHGSDLGKKLLAAARAGQLDEVRELIAAGADVNAKDYFSHTPLHLAARNGHLKIVEVLLKAGADVNAKDFAGKTPLHLAANEGHLEIVEVLLKAGADVNAQDIFGKTPADIAADAGHEDIAEVLQKAA

SEQ ID NO: 98 - protein, 24 aa, Artificial Sequence
  Synthetic construct
GSPTPTPTTPTPTPTTPTPTPTGS

SEQ ID NO: 99 - protein, 22 aa, Artificial Sequence
  Synthetic construct
GSPTPTPTTPTPTPTTPTPTPT

SEQ ID NO: 100 - protein, 5 aa, Artificial Sequence
  Synthetic construct
GGGGS